European Patent Application EP 4 538 288 A1, published April 16, 2025. Title: ANTI-CD40 ANTIBODY AND USE THEREOF. Applicant: BIOTHEUS INC. Application CN. The sequence listing filed with the application follows.

SEQUENCE LISTING (83 sequences)

SEQ ID NO: 1 - protein, 9 aa, synthetic construct
  source 1..9: note = VH CDR1
FTFSSYGMH

SEQ ID NO: 2 - protein, 9 aa, synthetic construct
  source 1..9: note = VH CDR1
FTFEKYGMH

SEQ ID NO: 3 - protein, 9 aa, synthetic construct
  source 1..9: note = VH CDR1
FTFGSYGMH

SEQ ID NO: 4 - protein, 9 aa, synthetic construct
  source 1..9: note = VH CDR1
FTFDDYAMH

SEQ ID NO: 5 - protein, 9 aa, synthetic construct
  source 1..9: note = VH CDR1
FTFDTYAMH

SEQ ID NO: 6 - protein, 9 aa, synthetic construct
  source 1..9: note = VH CDR1
GSISSYYWS

SEQ ID NO: 7 - protein, 11 aa, synthetic construct
  source 1..11: note = VL CDR1
  VARIANT 1: note = X is selected from (i) amino acid residues R, E; and (ii) amino acid residues that are conservative substitutions relative to (i).
  VARIANT 4: note = X is selected from (i) amino acid residues Q, K; and (ii) amino acid residues that are conservative substitutions relative to (i).
  VARIANT 5: note = X is selected from (i) amino acid residues G, V; and (ii) amino acid residues that are conservative substitutions relative to (i).
XASXXISSWLA

SEQ ID NO: 8 - skipped

SEQ ID NO: 9 - protein, 7 aa, synthetic construct
  source 1..7: note = VL CDR2
  VARIANT 4: note = X is selected from (i) amino acid residues S, Y; and (ii) amino acid residues that are conservative substitutions relative to (i).
  VARIANT 6: note = X is selected from (i) amino acid residues Q, E; and (ii) amino acid residues that are conservative substitutions relative to (i).
AASXLXS

SEQ ID NO: 10 - protein, 10 aa, synthetic construct
  source 1..10: note = VL CDR3
  VARIANT 1: note = X is selected from (i) amino acid residues S, Q, G; and (ii) amino acid residues that are conservative substitutions relative to (i).
  VARIANT 2: note = X is selected from (i) amino acid residues E, Q, D; and (ii) amino acid residues that are conservative substitutions relative to (i).
  VARIANT 4: note = X is selected from (i) amino acid residues A, S; and (ii) amino acid residues that are conservative substitutions relative to (i).
XXYXDYPPFT

SEQ ID NO: 11 - protein, 9 aa, synthetic construct
  source 1..9: note = VL CDR3
  VARIANT 3: note = X is selected from (i) amino acid residues R, H, V; and (ii) amino acid residues that are conservative substitutions relative to (i).
  VARIANT 4: note = X is selected from (i) amino acid residues S, L, A; and (ii) amino acid residues that are conservative substitutions relative to (i).
  VARIANT 6: note = X is selected from (i) amino acid residues F, Y; and (ii) amino acid residues that are conservative substitutions relative to (i).
QQXXSXPPT

SEQ ID NO: 12 - protein, 17 aa, synthetic construct
  source 1..17: note = VH CDR2
VISYEGSNKYYADSVKG

SEQ ID NO: 13 - protein, 17 aa, synthetic construct
  source 1..17: note = VH CDR2
VISYHASSKYYADSVKG

SEQ ID NO: 14 - protein, 17 aa, synthetic construct
  source 1..17: note = VH CDR2
VIHYEGSIKYYADSVKG

SEQ ID NO: 15 - protein, 17 aa, synthetic construct
  source 1..17: note = VH CDR2
VISYEGEKKYYADSVKG

SEQ ID NO: 16 - protein, 17 aa, synthetic construct
  source 1..17: note = VH CDR2
VISYEGTKKYYADSVKG

SEQ ID NO: 17 - protein, 17 aa, synthetic construct
  source 1..17: note = VH CDR2
VISYEGTSKYYADSVKG

SEQ ID NO: 18 - protein, 17 aa, synthetic construct
  source 1..17: note = VH CDR2
VISYEGVKKYYADSVKG

SEQ ID NO: 19 - protein, 17 aa, synthetic construct
  source 1..17: note = VH CDR2
GISWSSGSIGYADSVKG

SEQ ID NO: 20 - protein, 17 aa, synthetic construct
  source 1..17: note = VH CDR2
GISWSSDSIHYADSVKG

SEQ ID NO: 21 - protein, 17 aa, synthetic construct
  source 1..17: note = VH CDR2
GISWSSGSIHYADSVKG

SEQ ID NO: 22 - protein, 16 aa, synthetic construct
  source 1..16: note = VH CDR2
SIYYSGSTNYNPSLKS

SEQ ID NO: 23 - protein, 10 aa, synthetic construct
  source 1..10: note = VH CDR3
ARDTSRGHDI

SEQ ID NO: 24 - protein, 16 aa, synthetic construct
  source 1..16: note = VH CDR3
AKDPTATTGARGYFDL

SEQ ID NO: 25 - protein, 12 aa, synthetic construct
  source 1..12: note = VH CDR3
ARDANYYKWHPY

SEQ ID NO: 26 - protein, 117 aa, synthetic construct
  source 1..117: note = VH
QVQLVESGGGVVQPGRSLRLSCAASGFTFSSYGMHWVRQAPGKGLEWVAVISYEGSNKYYADSVKGRFTISRDNSKNTLYLQMNSLRAEDTAVYYCARDTSRGHDIWGQGTMVTVSS

SEQ ID NO: 27 - protein, 117 aa, synthetic construct
  source 1..117: note = VH
QVQLVESGGGVVQPGRSLRLSCAASGFTFSSYGMHWVRQAPGKGLEWVAVISYHASSKYYADSVKGRFTISRDNSKNTLYLQMNSLRAEDTAVYYCARDTSRGHDIWGQGTMVTVSS

SEQ ID NO: 28 - protein, 117 aa, synthetic construct
  source 1..117: note = VH
QVQLVESGGGVVQPGRSLRLSCAASGFTFEKYGMHWVRQAPGKGLEWVAVIHYEGSIKYYADSVKGRFTISRDNSKNTLYLQMNSLRAEDTAVYYCARDTSRGHDIWGQGTMVTVSS

SEQ ID NO: 29 - protein, 117 aa, synthetic construct
  source 1..117: note = VH
QVQLVESGGGVVQPGRSLRLSCAASGFTFEKYGMHWVRQAPGKGLEWVAVISYEGEKKYYADSVKGRFTISRDNSKNTLYLQMNSLRAEDTAVYYCARDTSRGHDIWGQGTMVTVSS

SEQ ID NO: 30 - protein, 117 aa, synthetic construct
  source 1..117: note = VH
QVQLVESGGGVVQPGRSLRLSCAASGFTFEKYGMHWVRQAPGKGLEWVAVISYEGTKKYYADSVKGRFTISRDNSKNTLYLQMNSLRAEDTAVYYCARDTSRGHDIWGQGTMVTVSS

SEQ ID NO: 31 - protein, 117 aa, synthetic construct
  source 1..117: note = VH
QVQLVESGGGVVQPGRSLRLSCAASGFTFEKYGMHWVRQAPGKGLEWVAVISYEGTSKYYADSVKGRFTISRDNSKNTLYLQMNSLRAEDTAVYYCARDTSRGHDIWGQGTMVTVSS

SEQ ID NO: 32 - protein, 117 aa, synthetic construct
  source 1..117: note = VH
QVQLVESGGGVVQPGRSLRLSCAASGFTFGSYGMHWVRQAPGKGLEWVAVISYEGVKKYYADSVKGRFTISRDNSKNTLYLQMNSLRAEDTAVYYCARDTSRGHDIWGQGTMVTVSS

SEQ ID NO: 33 - protein, 123 aa, synthetic construct
  source 1..123: note = VH
EVQLVESGGGLVQPGRSLRLSCAASGFTFDDYAMHWVRQAPGKGLEWVSGISWSSGSIGYADSVKGRFTISRDNAKNSLYLQMNSLRAEDTAVYYCAKDPTATTGARGYFDLWGRGTLVTVSS

SEQ ID NO: 34 - protein, 123 aa, synthetic construct
  source 1..123: note = VH
EVQLVESGGGLVQPGRSLRLSCAASGFTFDDYAMHWVRQAPGKGLEWVSGISWSSDSIHYADSVKGRFTISRDNAKNSLYLQMNSLRAEDTAVYYCAKDPTATTGARGYFDLWGRGTLVTVSS

SEQ ID NO: 35 - protein, 123 aa, synthetic construct
  source 1..123: note = VH
EVQLVESGGGLVQPGRSLRLSCAASGFTFDTYAMHWVRQAPGKGLEWVSGISWSSGSIHYADSVKGRFTISRDNAKNSLYLQMNSLRAEDTAVYYCAKDPTATTGARGYFDLWGRGTLVTVSS

SEQ ID NO: 36 - protein, 118 aa, synthetic construct
  source 1..118: note = VH
QVQLQESGPGLVKPSETLSLTCTVSGGSISSYYWSWIRQPPGKGLEWIGSIYYSGSTNYNPSLKSRVTISVDTSKNQFSLKLSSVTAADTAVYYCARDANYYKWHPYWGQGTLVTVSS

SEQ ID NO: 37 - protein, 12 aa, synthetic construct
  source 1..12: note = VL CDR1
RASQSVSSSYLA

SEQ ID NO: 38 - protein, 12 aa, synthetic construct
  source 1..12: note = VL CDR1
RASQSVSYDYLA

SEQ ID NO: 39 - protein, 12 aa, synthetic construct
  source 1..12: note = VL CDR1
RASQSVSYSYLA

SEQ ID NO: 40 - protein, 12 aa, synthetic construct
  source 1..12: note = VL CDR1
QASQSVSYNYLA

SEQ ID NO: 41 - protein, 11 aa, synthetic construct
  source 1..11: note = VL CDR1
RASQGISSWLA

SEQ ID NO: 42 - protein, 11 aa, synthetic construct
  source 1..11: note = VL CDR1
RASKVISSWLA

SEQ ID NO: 43 - protein, 11 aa, synthetic construct
  source 1..11: note = VL CDR1
EASQVISSWLA

SEQ ID NO: 44 - protein, 12 aa, synthetic construct
  source 1..12: note = VL CDR1
RASQSVSSDYLA

SEQ ID NO: 45 - protein, 7 aa, synthetic construct
  source 1..7: note = VL CDR2
GASSRAT

SEQ ID NO: 46 - protein, 7 aa, synthetic construct
  source 1..7: note = VL CDR2
GASTRAN

SEQ ID NO: 47 - protein, 7 aa, synthetic construct
  source 1..7: note = VL CDR2
GASSRAN

SEQ ID NO: 48 - protein, 7 aa, synthetic construct
  source 1..7: note = VL CDR2
GASSLAT

SEQ ID NO: 49 - protein, 7 aa, synthetic construct
  source 1..7: note = VL CDR2
GASSRNN

SEQ ID NO: 50 - protein, 7 aa, synthetic construct
  source 1..7: note = VL CDR2
GASARAN

SEQ ID NO: 51 - protein, 7 aa, synthetic construct
  source 1..7: note = VL CDR2
AASSLQS

SEQ ID NO: 52 - protein, 7 aa, synthetic construct
  source 1..7: note = VL CDR2
AASYLES

SEQ ID NO: 53 - protein, 7 aa, synthetic construct
  source 1..7: note = VL CDR2
AASYLQS

SEQ ID NO: 54 - protein, 10 aa, synthetic construct
  source 1..10: note = VL CDR3
QQYADYPPFT

SEQ ID NO: 55 - protein, 10 aa, synthetic construct
  source 1..10: note = VL CDR3
GEYADYPPFT

SEQ ID NO: 56 - protein, 10 aa, synthetic construct
  source 1..10: note = VL CDR3
SDYADYPPFT

SEQ ID NO: 57 - protein, 10 aa, synthetic construct
  source 1..10: note = VL CDR3
QQYSDYPPFT

SEQ ID NO: 58 - protein, 9 aa, synthetic construct
  source 1..9: note = VL CDR3
QQRASFPPT

SEQ ID NO: 59 - protein, 9 aa, synthetic construct
  source 1..9: note = VL CDR3
QQHSSFPPT

SEQ ID NO: 60 - protein, 9 aa, synthetic construct
  source 1..9: note = VL CDR3
QQVLSYPPT

SEQ ID NO: 61 - protein, 109 aa, synthetic construct
  source 1..109: note = VL
EIVLTQSPGTLSLSPGERATLSCRASQSVSSSYLAWYQQKPGQAPRLLIYGASSRATGIPDRFSGSGSGTDFTLTISRLEPEDFAVYYCQQYADYPPFTFGGGTKVEIK

SEQ ID NO: 62 - protein, 109 aa, synthetic construct
  source 1..109: note = VL
EIVLTQSPGTLSLSPGERATLSCRASQSVSYDYLAWYQQKPGQAPRLLIYGASTRANGIPDRFSGSGSGTDFTLTISRLEPEDFAVYYCGEYADYPPFTFGGGTKVEIK

SEQ ID NO: 63 - protein, 109 aa, synthetic construct
  source 1..109: note = VL
EIVLTQSPGTLSLSPGERATLSCRASQSVSYSYLAWYQQKPGQAPRLLIYGASSRANGIPDRFSGSGSGTDFTLTISRLEPEDFAVYYCSDYADYPPFTFGGGTKVEIK

SEQ ID NO: 64 - protein, 109 aa, synthetic construct
  source 1..109: note = VL
EIVLTQSPGTLSLSPGERATLSCRASQSVSYSYLAWYQQKPGQAPRLLIYGASSLATGIPDRFSGSGSGTDFTLTISRLEPEDFAVYYCQQYSDYPPFTFGGGTKVEIK

SEQ ID NO: 65 - protein, 109 aa, synthetic construct
  source 1..109: note = VL
EIVLTQSPGTLSLSPGERATLSCQASQSVSYNYLAWYQQKPGQAPRLLIYGASSRNNGIPDRFSGSGSGTDFTLTISRLEPEDFAVYYCQQYSDYPPFTFGGGTKVEIK

SEQ ID NO: 66 - protein, 109 aa, synthetic construct
  source 1..109: note = VL
EIVLTQSPGTLSLSPGERATLSCRASQSVSYDYLAWYQQKPGQAPRLLIYGASARANGIPDRFSGSGSGTDFTLTISRLEPEDFAVYYCQQYADYPPFTFGGGTKVEIK

SEQ ID NO: 67 - protein, 107 aa, synthetic construct
  source 1..107: note = VL
DIQMTQSPSSVSASVGDRVTITCRASQGISSWLAWYQQKPGKAPKLLIYAASSLQSGVPSRFSGSGSGTDFTLTISSLQPEDFATYYCQQRASFPPTFGGGTKVEIK

SEQ ID NO: 68 - protein, 107 aa, synthetic construct
  source 1..107: note = VL
DIQMTQSPSSVSASVGDRVTITCRASKVISSWLAWYQQKPGKAPKLLIYAASYLESGVPSRFSGSGSGTDFTLTISSLQPEDFATYYCQQHSSFPPTFGGGTKVEIK

SEQ ID NO: 69 - protein, 107 aa, synthetic construct
  source 1..107: note = VL
DIQMTQSPSSVSASVGDRVTITCEASQVISSWLAWYQQKPGKAPKLLIYAASYLQSGVPSRFSGSGSGTDFTLTISSLQPEDFATYYCQQHSSFPPTFGGGTKVEIK

SEQ ID NO: 70 - protein, 108 aa, synthetic construct
  source 1..108: note = VL
EIVLTQSPGTLSLSPGERATLSCRASQSVSSDYLAWYQQKPGQAPRLLIYGASSRATGIPDRFSGSGSGTDFTLTISRLEPEDFAVYYCQQVLSYPPTFGGGTKVEIK

SEQ ID NO: 71 - protein, 277 aa, synthetic construct
  source 1..277: note = human CD40
MVRLPLQCVLWGCLLTAVHPEPPTACREKQYLINSQCCSLCQPGQKLVSDCTEFTETECLPCGESEFLDTWNRETHCHQHKYCDPNLGLRVQQKGTSETDTICTCEEGWHCTSEACESCVLHRSCSPGFGVKQIATGVSDTICEPCPVGFFSNVSSAFEKCHPWTSCETKDLVVQQAGTNKTDVVCGPQDRLRALVVIPIIFGILFAILLVLVFIKKVAKKPTNKAPHPKQEPQEINFPDDLPGSNTAAPVQETLHGCQPVTQEDGKESRISVQERQ

SEQ ID NO: 72 - protein, 329 aa, synthetic construct
  source 1..329: note = the constant region of an antibody heavy chain
ASTKGPSVFPLAPSSKSTSGGTAALGCLVKDYFPEPVTVSWNSGALTSGVHTFPAVLQSSGLYSLSSVVTVPSSSLGTQTYICNVNHKPSNTKVDKKVEPKSCDKTHTCPPCPAPELLGGPSVFLFPPKPKDTLMISRTPEVTCVVVDVSHEDPEVKFNWYVDGVEVHNAKTKPREEQYNSTYRVVSVLTVLHQDWLNGKEYKCKVSNKALPAPIEKTISKAKGQPREPQVYTLPPSRDELTKNQVSLTCLVKGFYPSDIAVEWESNGQPENNYKTTPPVLDSDGSFFLYSKLTVDKSRWQQGNVFSCSVMHEALHNHYTQKSLSLSPG

SEQ ID NO: 73 - protein, 107 aa, synthetic construct [sequence omitted]

SEQ ID NO: 74 - protein, 239 aa, synthetic construct
  source 1..239: note = cynomolgus CD40
MVSKGEELFTGVVPILVELDGDVNGHKFSVSGEGEGDATYGKLTLKFICTTGKLPVPWPTLVTTLTYGVQCFSRYPDHMKKHDFFKSAMPEGYVQERTIFFKDDGNYKTRAEVKFEGDTLVNRIELKGIDFKEDGNILGHKLEYNYNSHNVYIMADKQKNGIKANFKVRHNIEDGSVQLADHYQQNTPIGDGPVLLPDNHYLSTQSALSKDPNEKRDHMVLLEFVTAAGITLGMDELYK

SEQ ID NO: 75 - protein, 261 aa, synthetic construct
  source 1..261: note = human CD40L
MIETYNQTSPRSAATGLPISMKIFMYLLTVFLITQMIGSALFAVYLHRRLDKIEDERNLHEDFVFMKTIQRCNTGERSLSLLNCEEIKSQFEGFVKDIMLNKEETKKENSFEMQKGDQNPQIAAHVISEASSKTTSVLQWAEKGYYTMSNNLVTLENGKQLTVKRQGLYYIYAQVTFCSNREASSQAPFIASLCLKSPGRFERILLRAANTHSSAKPCGQQSIHLGGVFELQPGASVFVNVTDPSQVSHGTGFTSFGLLKL

SEQ ID NO: 76 - protein, 9 aa, synthetic construct
  source 1..9: note = VH CDR1
  VARIANT 4: note = X is selected from (i) amino acid residues S, E, G, D; and (ii) amino acid residues that are conservative substitutions relative to (i).
  VARIANT 5: note = X is selected from (i) amino acid residues S, K, D, T; and (ii) amino acid residues that are conservative substitutions relative to (i).
  VARIANT 7: note = X is selected from (i) amino acid residues G, A; and (ii) amino acid residues that are conservative substitutions relative to (i).
FTFXXYXMH

SEQ ID NO: 77 - protein, 17 aa, synthetic construct
  source 1..17: note = VH CDR2
  VARIANT 3: note = X is selected from (i) amino acid residues S, H; and (ii) amino acid residues that are conservative substitutions relative to (i).
  VARIANT 5: note = X is selected from (i) amino acid residues E, H; and (ii) amino acid residues that are conservative substitutions relative to (i).
  VARIANT 6: note = X is selected from (i) amino acid residues G, A; and (ii) amino acid residues that are conservative substitutions relative to (i).
  VARIANT 7: note = X is selected from (i) amino acid residues S, E, T, V; and (ii) amino acid residues that are conservative substitutions relative to (i).
  VARIANT 8: note = X is selected from (i) amino acid residues N, S, I, K; and (ii) amino acid residues that are conservative substitutions relative to (i).
  VARIANT 13: note = X is selected from (i) amino acid residues D, E; and (ii) amino acid residues that are conservative substitutions relative to (i).
VIXYXXXXKYYAXSVKG

SEQ ID NO: 78 - protein, 17 aa, synthetic construct
  source 1..17: note = VH CDR2
  VARIANT 7: note = X is selected from (i) amino acid residues G, D; and (ii) amino acid residues that are conservative substitutions relative to (i).
  VARIANT 10: note = X is selected from (i) amino acid residues G, H; and (ii) amino acid residues that are conservative substitutions relative to (i).
GISWSSXSIXYADSVKG

SEQ ID NO: 79 - protein, 12 aa, synthetic construct
  source 1..12: note = VL CDR1
  VARIANT 1: note = X is selected from (i) amino acid residues R, Q; and (ii) amino acid residues that are conservative substitutions relative to (i).
  VARIANT 8: note = X is selected from (i) amino acid residues Y, S; and (ii) amino acid residues that are conservative substitutions relative to (i).
  VARIANT 9: note = X is selected from (i) amino acid residues S, D, N; and (ii) amino acid residues that are conservative substitutions relative to (i).
XASQSVSXXYLA

SEQ ID NO: 80 - protein, 234 aa, synthetic construct
  source 1..234: note = the light chain of CP870893-IgG2
MRLPAQLLGLLLLWFPGSRCDIQMTQSPSSVSASVGDRVTITCRASQGIYSWLAWYQQKPGKAPNLLIYTASTLQSGVPSRFSGSGSGTDFTLTISSLQPEDFATYYCQQANIFPLTFGGGTKVEIKRTVAAPSVFIFPPSDEQLKSGTASVVCLLNNFYPREAKVQWKVDNALQSGNSQESVTEQDSKDSTYSLSSTLTLSKADYEKHKVYACEVTHQGLSSPVTKSFNRGEC

SEQ ID NO: 81 - protein, 471 aa, synthetic construct
  source 1..471: note = the heavy chain of CP870893-IgG2
MDWTWRILFLVAAATGAHSQVQLVQSGAEVKKPGASVKVSCKASGYTFTGYYMHWVRQAPGQGLEWMGWINPDSGGTNYAQKFQGRVTMTRDTSISTAYMELNRLRSDDTAVYYCARDQPLGYCTNGVCSYFDYWGQGTLVTVSSASTKGPSVFPLAPCSRSTSESTAALGCLVKDYFPEPVTVSWNSGALTSGVHTFPAVLQSSGLYSLSSVVTVPSSNFGTQTYTCNVDHKPSNTKVDKTVERKCCVECPPCPAPPVAGPSVFLFPPKPKDTLMISRTPEVTCVVVDVSHEDPEVQFNWYVDGVEVHNAKTKPREEQFNSTFRVVSVLTVVHQDWLNGKEYKCKVSNKGLPAPIEKTISKTKGQPREPQVYTLPPSREEMTKNQVSLTCLVKGFYPSDIAVEWESNGQPENNYKTTPPMLDSDGSFFLYSKLTVDKSRWQQGNVFSCSVMHEALHNHYTQKSLSLSPGK

SEQ ID NO: 82 - protein, 17 aa, synthetic construct
  source 1..17: note = VH CDR2
VISYEGTKKYYAESVKG

SEQ ID NO: 83 - protein, 117 aa, synthetic construct
  source 1..117: note = VH
QVQLVESGGGVVQPGRSLRLSCAASGFTFEKYGMHWVRQAPGKGLEWVAVISYEGTKKYYAESVKGRFTISRDNSKNTLYLQMNSLRAEDTAVYYCARDTSRGHDIWGQGTMVTVSS